European Patent Application EP 4 527 851 A1, published March 26, 2025. Title: Bispecific antibodies (BsAB) binding LTβR and LRRC15. Applicant: Bayer Aktiengesellschaft. Application EP. The sequence listing filed with the application follows.

SEQUENCE LISTING (152 sequences)

SEQ ID NO: 1 - protein, 715 aa, synthetic construct
EVQLVQSGAEVKKPGASVKVSCKASGYKFSSYWIEWVKQAPGQGLEWIGEILPGSDTTNYNEKFKDRATFTSDTSINTAYMELSRLRSDDTAVYYCARDRGNYRAWFGYWGQGTLVTVSSASTKGPSVFPLAPSSKSTSGGTAALGCLVKDYFPEPVTVSWNSGALTSGVHTFPAVLQSSGLYSLSSVVTVPSSSLGTQTYICNVNHKPSNTKVDKKVEPKSCDKTHTCPPCPAPPVAGPSVFLFPPKPKDTLMISRTPEVTCVVVGVSHEDPEVKFNWYVDGVEVHNAKTKPREEQYNSTYRVVSVLTVLHQDWLNGKEYKCKVSNKQLPSPIEKTISKAKGQPREPQVYTLPPSRDELTKNQVSLTCLVKGFYPSDIAVEWESNGQPENNYKTTPPVLDSDGSFFLYSKLTVDKSRWQQGNVFSCSVMHEALHNHYTQKSLSLSPGGGGGSGGSGGSGGGGGEVQLLESGGGLVQPGGSLRLSCAASGFTFSDHYMDWVRQAPGKGLEWVAVIWYDGSNKYYADSVKGRFTISRDNSKNTLYLQMNSLRAEDTAVYYCARRPRGYYYYGMDVWGQGTLVTVSSGGGGSGGGGSGGGGSGGGGSQSVLTQPPSASGTPGQRVTISCSGGSSNVGSNPVNWYQQLPGTAPKLLIYGNTNRPSGVPDRFSGSKSGTSASLAISGLRSEDEADYYCAAWDASLSGWVFGGGTKLTVL

SEQ ID NO: 2 - protein, 214 aa, synthetic construct
DIQMTQSPSSLSASVGDRVTITCRASQSISSYLNWYQQKPGGAPKFLIYYASSLQSGVPSRFSGSGSGTDYTLTISSLQPEDFATYYCQQGFSLPWTFGGGTKVEIKRTVAAPSVFIFPPSDEQLKSGTASVVCLLNNFYPREAKVQWKVDNALQSGNSQESVTEQDSKDSTYSLSSTLTLSKADYEKHKVYACEVTHQGLSSPVTKSFNRGEC

SEQ ID NO: 3 - protein, 716 aa, synthetic construct
EVQLVQSGAEVKKPGASVKVSCKASGYKFSSYWIEWVKQAPGQGLEWIGEILPGSDTTNYNEKFKDRATFTSDTSINTAYMELSRLRSDDTAVYYCARDRGNYRAWFGYWGQGTLVTVSSASTKGPSVFPLAPSSKSTSGGTAALGCLVKDYFPEPVTVSWNSGALTSGVHTFPAVLQSSGLYSLSSVVTVPSSSLGTQTYICNVNHKPSNTKVDKKVEPKSCDKTHTCPPCPAPELLGGPSVFLFPPKPKDTLMISRTPEVTCVVVDVSHEDPEVKFNWYVDGVEVHNAKTKPREEQYNSTYRVVSVLTVLHQDWLNGKEYKCKVSNKALPAPIEKTISKAKGQPREPQVYTLPPSRDELTKNQVSLTCLVKGFYPSDIAVEWESNGQPENNYKTTPPVLDSDGSFFLYSKLTVDKSRWQQGNVFSCSVMHEALHNHYTQKSLSLSPGGGGGSGGSGGSGGGGGEVQLLESGGGLVQPGGSLRLSCAASGFTFSDHYMDWVRQAPGKGLEWVAVIWYDGSNKYYADSVKGRFTISRDNSKNTLYLQMNSLRAEDTAVYYCARRPRGYYYYGMDVWGQGTLVTVSSGGGGSGGGGSGGGGSGGGGSQSVLTQPPSASGTPGQRVTISCSGGSSNVGSNPVNWYQQLPGTAPKLLIYGNTNRPSGVPDRFSGSKSGTSASLAISGLRSEDEADYYCAAWDASLSGWVFGGGTKLTVL

SEQ ID NO: 4 - protein, 214 aa, synthetic construct; identical to SEQ ID NO: 2

SEQ ID NO: 5 - protein, 712 aa, synthetic construct
EVQLVQSGAEVKKPGASVKVSCKASGYKFSSYWIEWVKQAPGQGLEWIGEILPGSDTTNYNEKFKDRATFTSDTSINTAYMELSRLRSDDTAVYYCARDRGNYRAWFGYWGQGTLVTVSSASTKGPSVFPLAPCSRSTSESTAALGCLVKDYFPEPVTVSWNSGALTSGVHTFPAVLQSSGLYSLSSVVTVPSSSLGTKTYTCNVDHKPSNTKVDKRVESKYGPPCPPCPAPEFLGGPSVFLFPPKPKDTLMISRTPEVTCVVVDVSQEDPEVQFNWYVDGVEVHNAKTKPREEQFNSTYRVVSVLTVLHQDWLNGKEYKCKVSNKGLPSSIEKTISKAKGQPREPQVYTLPPSQEEMTKNQVSLTCLVKGFYPSDIAVEWESNGQPENNYKTTPPVLDSDGSFFLYSRLTVDKSRWQEGNVFSCSVMHEALHNHYTQKSLSLSLGGGGGSGGSGGSGGGGGEVQLLESGGGLVQPGGSLRLSCAASGFTFSSYGIHWVRQAPGKGLEWVAVIPYDGSNKYYADSVKGRFTISRDNSKNTLYLQMNSLRAEDTAVYYCARDPWGYDYGLDVWGQGTLVTVSSGGGGSGGGGSGGGGSGGGGSQSVLTQPPSASGTPGQRVTISCSGGASNIETNYVSWYQQLPGTAPKLLIYDNNRRPSGVPDRFSGSKSGTSASLAISGLRSEDEADYYCAAWDDSLNGVIFGGGTKLTVL

SEQ ID NO: 6 - protein, 214 aa, synthetic construct; identical to SEQ ID NO: 2

SEQ ID NO: 7 - protein, 713 aa, synthetic construct
EVQLVQSGAEVKKPGASVKVSCKASGYKFSSYWIEWVKQAPGQGLEWIGEILPGSDTTNYNEKFKDRATFTSDTSINTAYMELSRLRSDDTAVYYCARDRGNYRAWFGYWGQGTLVTVSSASTKGPSVFPLAPCSRSTSESTAALGCLVKDYFPEPVTVSWNSGALTSGVHTFPAVLQSSGLYSLSSVVTVPSSSLGTKTYTCNVDHKPSNTKVDKRVESKYGPPCPPCPAPEFLGGPSVFLFPPKPKDTLMISRTPEVTCVVVDVSQEDPEVQFNWYVDGVEVHNAKTKPREEQFNSTYRVVSVLTVLHQDWLNGKEYKCKVSNKGLPSSIEKTISKAKGQPREPQVYTLPPSQEEMTKNQVSLTCLVKGFYPSDIAVEWESNGQPENNYKTTPPVLDSDGSFFLYSRLTVDKSRWQEGNVFSCSVMHEALHNHYTQKSLSLSLGGGGGSGGSGGSGGGGGEVQLLESGGGLVQPGGSLRLSCAASGFTFSDHYMDWVRQAPGKGLEWVAVIWYDGSNKYYADSVKGRFTISRDNSKNTLYLQMNSLRAEDTAVYYCARRPRGYYYYGMDVWGQGTLVTVSSGGGGSGGGGSGGGGSGGGGSQSVLTQPPSASGTPGQRVTISCSGGSSNVGSNPVNWYQQLPGTAPKLLIYGNTNRPSGVPDRFSGSKSGTSASLAISGLRSEDEADYYCAAWDASLSGWVFGGGTKLTVL

SEQ ID NO: 8 - protein, 214 aa, synthetic construct; identical to SEQ ID NO: 2

SEQ ID NO: 9 - protein, 711 aa, synthetic construct
EVQLVQSGAEVKKPGASVKVSCKASGYKFSSYWIEWVKQAPGQGLEWIGEILPGSDTTNYNEKFKDRATFTSDTSINTAYMELSRLRSDDTAVYYCARDRGNYRAWFGYWGQGTLVTVSSAKTTPPSVYPLAPGSAAQTNSMVTLGCLVKGYFPEPVTVTWNSGSLSSGVHTFPAVLQSDLYTLSSSVTVPSSTWPSETVTCNVAHPASSTKVDKKIVPRDCGCKPCICTVPEVSSVFIFPPKPKDVLTITLTPKVTCVVVDISKDDPEVQFSWFVDDVEVHTAQTQPREEQFASTFRSVSELPIMHQDWLNGKEFKCRVNSAAFPAPIEKTISKTKGRPKAPQVYTIPPPKEQMAKDKVSLTCMITDFFPEDITVEWQWNGQPAENYKNTQPIMDTDGSYFVYSKLNVQKSNWEAGNTFTCSVLHEGLHNHHTEKSLSHSPGKGGGGSGGSGGSGGGGGEVQLLESGGGLVQPGGSLRLSCAASGFTFSDHYMDWVRQAPGKGLEWVAVIWYDGSNKYYADSVKGRFTISRDNSKNTLYLQMNSLRAEDTAVYYCARRPRGYYYYGMDVWGQGTLVTVSSGGGGSGGGGSGGGGSGGGGSQSVLTQPPSASGTPGQRVTISCSGGSSNVGSNPVNWYQQLPGTAPKLLIYGNTNRPSGVPDRFSGSKSGTSASLAISGLRSEDEADYYCAAWDASLSGWVFGGGTKLTVL

SEQ ID NO: 10 - protein, 214 aa, synthetic construct
DIQMTQSPSSLSASVGDRVTITCRASQSISSYLNWYQQKPGGAPKFLIYYASSLQSGVPSRFSGSGSGTDYTLTISSLQPEDFATYYCQQGFSLPWTFGGGTKVEIKRADAAPTVSIFPPSSEQLTSGGASVVCFLNNFYPKDINVKWKIDGSERQNGVLNSWTDQDSKDSTYSMSSTLTLTKDEYERHNSYTCEATHKTSTSPIVKSFNRNEC

SEQ ID NO: 11 - protein, 713 aa, synthetic construct
EVQLVQSGAEVKKPGASVKVSCKASGYKFSSYWIEWVKQAPGQGLEWIGEILPGSDTTNYNEKFKDRATFTSDTSINTAYMELSRLRSDDTAVYYCARDRGNYRAWFGYWGQGTLVTVSSASTKGPSVFPLAPCSRSTSESTAALGCLVKDYFPEPVTVSWNSGALTSGVHTFPAVLQSSGLYSLSSVVTVPSSSLGTKTYTCNVDHKPSNTKVDKRVESKYGPPCPPCPAPEFLGGPSVFLFPPKPKDTLMISRTPEVTCVVVDVSQEDPEVQFNWYVDGVEVHNAKTKPREEQFNSTYRVVSVLTVLHQDWLNGKEYKCKVSNKGLPSSIEKTISKAKGQPREPQVYTLPPSQEEMTKNQVSLTCLVKGFYPSDIAVEWESNGQPENNYKTTPPVLDSDGSFFLYSRLTVDKSRWQEGNVFSCSVMHEALHNHYTQKSLSLSLGGGGGSGGSGGSGGGGGQVQLVESGGGLVQPGGSLRLSCAASGFTFSDHYMDWVRQAPGKGLEWVAVIWYDGSNKYYADSVKGRFTISRDNSKNTLYLQMNSLRAEDTAVYYCARRPRGYYYYGMDVWGQGTLVTVSSGGGGSGGGGSGGGGSGGGGSQSVLTQPPSASGTPGQRVTISCSGGSSNIGSNPVNWYQQLPGTAPKLLIYGNTQRPSGVPDRFSGSKSGTSASLAISGLRSEDEADYYCAAWDDSLSGWVFGGGTKLTVL

SEQ ID NO: 12 - protein, 214 aa, synthetic construct; identical to SEQ ID NO: 2

SEQ ID NO: 13 - protein, 716 aa, synthetic construct
EVQLVQSGAEVKKPGASVKVSCKASGYKFSSYWIEWVKQAPGQGLEWIGEILPGSDTTNYNEKFKDRATFTSDTSINTAYMELSRLRSDDTAVYYCARDRGNYRAWFGYWGQGTLVTVSSASTKGPSVFPLAPSSKSTSGGTAALGCLVKDYFPEPVTVSWNSGALTSGVHTFPAVLQSSGLYSLSSVVTVPSSSLGTQTYICNVNHKPSNTKVDKKVEPKSCDKTHTCPPCPAPEAAGGPSVFLFPPKPKDTLMISRTPEVTCVVVDVSHEDPEVKFNWYVDGVEVHNAKTKPREEQYNSTYRVVSVLTVLHQDWLNGKEYKCKVSNKALPAPIEKTISKAKGQPREPQVYTLPPSRDELTKNQVSLTCLVKGFYPSDIAVEWESNGQPENNYKTTPPVLDSDGSFFLYSKLTVDKSRWQQGNVFSCSVMHEALHNHYTQKSLSLSPGGGGGSGGSGGSGGGGGQVQLVESGGGLVQPGGSLRLSCAASGFTFSDHYMDWVRQAPGKGLEWVAVIWYDGSNKYYADSVKGRFTISRDNSKNTLYLQMNSLRAEDTAVYYCARRPRGYYYYGMDVWGQGTLVTVSSGGGGSGGGGSGGGGSGGGGSQSVLTQPPSASGTPGQRVTISCSGGSSNIGSNPVNWYQQLPGTAPKLLIYGNTQRPSGVPDRFSGSKSGTSASLAISGLRSEDEADYYCAAWDDSLSGWVFGGGTKLTVL

SEQ ID NO: 14 - protein, 214 aa, synthetic construct; identical to SEQ ID NO: 2

SEQ ID NO: 15 - protein, 716 aa, synthetic construct
EVQLVQSGAEVKKPGASVKVSCKASGYKFSSYWIEWVKQAPGQGLEWIGEILPGSDTTNYNEKFKDRATFTSDTSINTAYMELSRLRSDDTAVYYCARDRGNYRAWFGYWGQGTLVTVSSASTKGPSVFPLAPSSKSTSGGTAALGCLVKDYFPEPVTVSWNSGALTSGVHTFPAVLQSSGLYSLSSVVTVPSSSLGTQTYICNVNHKPSNTKVDKKVEPKSCDKTHTCPPCPAPEAAGGPSVFLFPPKPKDTLMISRTPEVTCVVVDVSHEDPEVKFNWYVDGVEVHNAKTKPREEQYNSTYRVVSVLTVLHQDWLNGKEYKCKVSNKALPAPIEKTISKAKGQPREPQVYTLPPSRDELTKNQVSLTCLVKGFYPSDIAVEWESNGQPENNYKTTPPVLDSDGSFFLYSKLTVDKSRWQQGNVFSCSVMHEALHNHYTQKSLSLSPGGGGGSGGSGGSGGGGGQVQLVESGGGLVQPGGSLRLSCAASGFTFSDHYMDWVRQAPGKGLEWVAVIWYDGSNKYYADSVKGRFTISRDNSKNTLYLQMNSLRAEDTAVYYCARRPRGYYYYGTDVWGQGTLVTVSSGGGGSGGGGSGGGGSGGGGSQSVLTQPPSASGTPGQRVTISCSGGSSNIGSNPVNWYQQLPGTAPKLLIYGNTQRPSGVPDRFSGSKSGTSASLAISGLRSEDEADYYCAAWDDSLSGWVFGGGTKLTVL

SEQ ID NO: 16 - protein, 214 aa, synthetic construct; identical to SEQ ID NO: 2

SEQ ID NO: 17 - protein, 711 aa, synthetic construct
EVQLVQSGAEVKKPGASVKVSCKASGYKFSSYWIEWVKQAPGQGLEWIGEILPGSDTTNYNEKFKDRATFTSDTSINTAYMELSRLRSDDTAVYYCARDRGNYRAWFGYWGQGTLVTVSSAKTTPPSVYPLAPGSAAQTNSMVTLGCLVKGYFPEPVTVTWNSGSLSSGVHTFPAVLQSDLYTLSSSVTVPSSTWPSETVTCNVAHPASSTKVDKKIVPRDCGCKPCICTVPEVSSVFIFPPKPKDVLTITLTPKVTCVVVDISKDDPEVQFSWFVDDVEVHTAQTQPREEQFASTFRSVSELPIMHQDWLNGKEFKCRVNSAAFPAPIEKTISKTKGRPKAPQVYTIPPPKEQMAKDKVSLTCMITDFFPEDITVEWQWNGQPAENYKNTQPIMDTDGSYFVYSKLNVQKSNWEAGNTFTCSVLHEGLHNHHTEKSLSHSPGKGGGGSGGSGGSGGGGGQVQLVESGGGLVQPGGSLRLSCAASGFTFSDHYMDWVRQAPGKGLEWVAVIWYDGSNKYYADSVKGRFTISRDNSKNTLYLQMNSLRAEDTAVYYCARRPRGYYYYGTDVWGQGTLVTVSSGGGGSGGGGSGGGGSGGGGSQSVLTQPPSASGTPGQRVTISCSGGSSNIGSNPVNWYQQLPGTAPKLLIYGNTQRPSGVPDRFSGSKSGTSASLAISGLRSEDEADYYCAAWDDSLSGWVFGGGTKLTVL

SEQ ID NO: 18 - protein, 214 aa, synthetic construct; identical to SEQ ID NO: 10

SEQ ID NO: 19 - protein, 715 aa, synthetic construct
EVQLVQSGAEVKKPGASVKVSCKASGYKFSSYWIEWVKQAPGQGLEWIGEILPGSDTTNYNEKFKDRATFTSDTSINTAYMELSRLRSDDTAVYYCARDRGNYRAWFGYWGQGTLVTVSSASTKGPSVFPLAPSSKSTSGGTAALGCLVKDYFPEPVTVSWNSGALTSGVHTFPAVLQSSGLYSLSSVVTVPSSSLGTQTYICNVNHKPSNTKVDKKVEPKSCDKTHTCPPCPAPPVAGPSVFLFPPKPKDTLMISRTPEVTCVVVGVSHEDPEVKFNWYVDGVEVHNAKTKPREEQYNSTYRVVSVLTVLHQDWLNGKEYKCKVSNKQLPSPIEKTISKAKGQPREPQVYTLPPSRDELTKNQVSLTCLVKGFYPSDIAVEWESNGQPENNYKTTPPVLDSDGSFFLYSKLTVDKSRWQQGNVFSCSVMHEALHNHYTQKSLSLSPGGGGGSGGSGGSGGGGGQVQLVESGGGLVQPGGSLRLSCAASGFTFSDHYMDWVRQAPGKGLEWVAVIWYDGSNKYYADSVKGRFTISRDNSKNTLYLQMNSLRAEDTAVYYCARRPRGYYYYGTDVWGQGTLVTVSSGGGGSGGGGSGGGGSGGGGSQSVLTQPPSASGTPGQRVTISCSGGSSNIGSNPVNWYQQLPGTAPKLLIYGNTQRPSGVPDRFSGSKSGTSASLAISGLRSEDEADYYCAAWDDSLSGWVFGGGTKLTVL

SEQ ID NO: 20 - protein, 214 aa, synthetic construct; identical to SEQ ID NO: 2

SEQ ID NO: 21 - protein, 715 aa, synthetic construct
EVQLVQSGAEVKKPGASVKVSCKASGYKFSSYWIEWVKQAPGQGLEWIGEILPGSDWTNYNEKFKDRATFTSDTSINTAYMELSRLRSDDTAVYYCARDRGNYRAWFQYWGQGTLVTVSSASTKGPSVFPLAPSSKSTSGGTAALGCLVKDYFPEPVTVSWNSGALTSGVHTFPAVLQSSGLYSLSSVVTVPSSSLGTQTYICNVNHKPSNTKVDKKVEPKSCDKTHTCPPCPAPPVAGPSVFLFPPKPKDTLMISRTPEVTCVVVGVSHEDPEVKFNWYVDGVEVHNAKTKPREEQYNSTYRVVSVLTVLHQDWLNGKEYKCKVSNKQLPSPIEKTISKAKGQPREPQVYTLPPSRDELTKNQVSLTCLVKGFYPSDIAVEWESNGQPENNYKTTPPVLDSDGSFFLYSKLTVDKSRWQQGNVFSCSVMHEALHNHYTQKSLSLSPGGGGGSGGSGGSGGGGGQVQLVESGGGLVQPGGSLRLSCAASGFTFSDHYMDWVRQAPGKGLEWVAVIWYDGSNKYYADSVKGRFTISRDNSKNTLYLQMNSLRAEDTAVYYCARRPRGYYYYGTDVWGQGTLVTVSSGGGGSGGGGSGGGGSGGGGSQSVLTQPPSASGTPGQRVTISCSGGSSNIGSNPVNWYQQLPGTAPKLLIYGNTQRPSGVPDRFSGSKSGTSASLAISGLRSEDEADYYCAAWDDSLSGWVFGGGTKLTVL

SEQ ID NO: 22 - protein, 214 aa, synthetic construct
DIQMTQSPSSLSASVGDRVTITCRASQSISSYLNWYQQKPGGAPKFLIYYASSLQSGVPSRFSGSGSGTDYTLTISSLQPEDFATYYCQQGLELPWTFGGGTKVEIKRTVAAPSVFIFPPSDEQLKSGTASVVCLLNNFYPREAKVQWKVDNALQSGNSQESVTEQDSKDSTYSLSSTLTLSKADYEKHKVYACEVTHQGLSSPVTKSFNRGEC

SEQ ID NO: 23 - protein, 443 aa, synthetic construct
EVQLVQSGAEVKKPGASVKVSCKASGYKFSSYWIEWVKQAPGQGLEWIGEILPGSDTTNYNEKFKDRATFTSDTSINTAYMELSRLRSDDTAVYYCARDRGNYRAWFGYWGQGTLVTVSSAKTTPPSVYPLAPGSAAQTNSMVTLGCLVKGYFPEPVTVTWNSGSLSSGVHTFPAVLQSDLYTLSSSVTVPSSTWPSETVTCNVAHPASSTKVDKKIVPRDCGCKPCICTVPEVSSVFIFPPKPKDVLTITLTPKVTCVVVDISKDDPEVQFSWFVDDVEVHTAQTQPREEQFASTFRSVSELPIMHQDWLNGKEFKCRVNSAAFPAPIEKTISKTKGRPKAPQVYTIPPPKEQMAKDKVSLTCMITDFFPEDITVEWQWNGQPAENYKNTQPIMDTDGSYFVYSKLNVQKSNWEAGNTFTCSVLHEGLHNHHTEKSLSHSPG

SEQ ID NO: 24 - protein, 465 aa, synthetic construct
DIQMTQSPSSLSASVGDRVTITCRASQSISSYLNWYQQKPGGAPKFLIYYASSLQSGVPSRFSGSGSGTDYTLTISSLQPEDFATYYCQQGFSLPWTFGGGTKVEIKRTVAAPSVFIFPPSDEQLKSGTASVVCLLNNFYPREAKVQWKVDNALQSGNSQESVTEQDSKDSTYSLSSTLTLSKADYEKHKVYACEVTHQGLSSPVTKSFNRGECGEVQLLESGGGLVQPGGSLRLSCAASGFTFSDHYMDWVRQAPGKGLEWVAVIWYDGSNKYYADSVKGRFTISRDNSKNTLYLQMNSLRAEDTAVYYCARRPRGYYYYGMDVWGQGTLVTVSGGGGSGGGGSGGGGSGGGGSQSVLTQPPSASGTPGQRVTISCSGGSSNVGSNPVNWYQQLPGTAPKLLIYGNTNRPSGVPDRFSGSKSGTSASLAISGLRSEDEADYYCAAWDASLSGWVFGGGTKLTVL

SEQ ID NO: 25 - protein, 712 aa, synthetic construct
EVQLVQSGAEVKKPGASVKVSCKASGYKFSSYWIEWVKQAPGQGLEWIGEILPGSDTTNYNEKFKDRATFTSDTSINTAYMELSRLRSDDTAVYYCARDRGNYRAWFGYWGQGTLVTVSSASTKGPSVFPLAPCSRSTSESTAALGCLVKDYFPEPVTVSWNSGALTSGVHTFPAVLQSSGLYSLSSVVTVPSSSLGTKTYTCNVDHKPSNTKVDKRVESKYGPPCPPCPAPEFLGGPSVFLFPPKPKDTLMISRTPEVTCVVVDVSQEDPEVQFNWYVDGVEVHNAKTKPREEQFNSTYRVVSVLTVLHQDWLNGKEYKCKVSNKGLPSSIEKTISKAKGQPREPQVYTLPPSQEEMTKNQVSLTCLVKGFYPSDIAVEWESNGQPENNYKTTPPVLDSDGSFFLYSRLTVDKSRWQEGNVFSCSVMHEALHNHYTQKSLSLSLGGGGGSGGSGGSGGGGGQVQLVESGGGVVQPGGSLRLSCAASGFTFSSYGMHWVRQAPGKGLEWVAVIPYDGSNKYYADSVKGRFTISRDNSKNTLYLQMNSLRAEDTAVYYCARDPWGYDYGLDVWGQGTTVTVSSGGGGSGGGGSGGGGSGGGGSQSVLTQPPSASGTPGQRVTISCSGGASNIGSNYVSWYQQLPGTAPKLLIYDNNQRPSGVPDRFSGSKSGTSASLAISGLRSEDEADYYCAAWDDSLSGVVFGGGTKLTVL

SEQ ID NO: 26 - protein, 214 aa, synthetic construct; identical to SEQ ID NO: 2

SEQ ID NO: 27 - protein, 17 aa, synthetic construct
GGGGGSGGSGGSGGGGG

SEQ ID NO: 28 - protein, 20 aa, synthetic construct
GGGGSGGGGSGGGGSGGGGS

SEQ ID NO: 29 - protein, 5 aa, synthetic construct
DHYMD

SEQ ID NO: 30 - protein, 17 aa, synthetic construct
VIWYDGSNKYYADSVKG

SEQ ID NO: 31 - protein, 12 aa, synthetic construct
RPRGYYYYGMDV

SEQ ID NO: 32 - protein, 13 aa, synthetic construct
SGGSSNVGSNPVN

SEQ ID NO: 33 - protein, 7 aa, synthetic construct
GNTNRPS

SEQ ID NO: 34 - protein, 11 aa, synthetic construct
AAWDASLSGWV

SEQ ID NO: 35 - protein, 121 aa, synthetic construct
EVQLLESGGGLVQPGGSLRLSCAASGFTFSDHYMDWVRQAPGKGLEWVAVIWYDGSNKYYADSVKGRFTISRDNSKNTLYLQMNSLRAEDTAVYYCARRPRGYYYYGMDVWGQGTLVTVSS

SEQ ID NO: 36 - protein, 110 aa, synthetic construct
QSVLTQPPSASGTPGQRVTISCSGGSSNVGSNPVNWYQQLPGTAPKLLIYGNTNRPSGVPDRFSGSKSGTSASLAISGLRSEDEADYYCAAWDASLSGWVFGGGTKLTVL

SEQ ID NO: 37 - protein, 251 aa, synthetic construct
EVQLLESGGGLVQPGGSLRLSCAASGFTFSDHYMDWVRQAPGKGLEWVAVIWYDGSNKYYADSVKGRFTISRDNSKNTLYLQMNSLRAEDTAVYYCARRPRGYYYYGMDVWGQGTLVTVSSGGGGSGGGGSGGGGSGGGGSQSVLTQPPSASGTPGQRVTISCSGGSSNVGSNPVNWYQQLPGTAPKLLIYGNTNRPSGVPDRFSGSKSGTSASLAISGLRSEDEADYYCAAWDASLSGWVFGGGTKLTVL

SEQ ID NO: 38 - DNA, 753 bp, synthetic construct
  source 1..753: mol_type = other DNA
gaagtgcagctgctggaatctggcggaggactggttcaacctggcggctctctgagactgtcttgtgccgccagcggcttcaccttcagcgaccactatatggactgggtccgacaggcccctggcaaaggacttgaatgggtcgccgtgatttggtacgacggcagcaacaagtactacgccgacagcgtgaagggcagattcaccatcagccgggacaacagcaagaacaccctgtacctgcagatgaacagcctgagagccgaggacaccgccgtgtactattgtgccagaaggcccagaggctactactactatggcatggacgtgtggggccagggcacactggttacagtttctagcggaggcggaggttctggcggcggaggaagtggtggcggaggctcaggtggcggtggatctcaatctgtgctgacccagcctcctagcgcctctggaacacctggacagagagtgaccatcagctgtagcggcggcagcagcaatgtgggcagcaaccccgtgaactggtatcagcagctccctggcacagcccctaaactgctgatctacggcaacaccaacagacccagcggcgtgcccgatagattttccggctctaagagcggcacctctgccagcctggctatctctggactgagaagcgaggacgaggccgactattactgtgccgcctgggatgcctctctgagcggatgggttttcggcggaggcaccaaactgacagtgctg

SEQ ID NO: 39 - protein, 5 aa, synthetic construct
SYGIH

SEQ ID NO: 40 - protein, 17 aa, synthetic construct
VIPYDGSNKYYADSVKG

SEQ ID NO: 41 - protein, 11 aa, synthetic construct
DPWGYDYGLDV

SEQ ID NO: 42 - protein, 13 aa, synthetic construct
SGGASNIETNYVS

SEQ ID NO: 43 - protein, 7 aa, synthetic construct
DNNRRPS

SEQ ID NO: 44 - protein, 11 aa, synthetic construct
AAWDDSLNGVI

SEQ ID NO: 45 - protein, 120 aa, synthetic construct
EVQLLESGGGLVQPGGSLRLSCAASGFTFSSYGIHWVRQAPGKGLEWVAVIPYDGSNKYYADSVKGRFTISRDNSKNTLYLQMNSLRAEDTAVYYCARDPWGYDYGLDVWGQGTLVTVSS

SEQ ID NO: 46 - protein, 110 aa, synthetic construct
QSVLTQPPSASGTPGQRVTISCSGGASNIETNYVSWYQQLPGTAPKLLIYDNNRRPSGVPDRFSGSKSGTSASLAISGLRSEDEADYYCAAWDDSLNGVIFGGGTKLTVL

SEQ ID NO: 47 - protein, 250 aa, synthetic construct
EVQLLESGGGLVQPGGSLRLSCAASGFTFSSYGIHWVRQAPGKGLEWVAVIPYDGSNKYYADSVKGRFTISRDNSKNTLYLQMNSLRAEDTAVYYCARDPWGYDYGLDVWGQGTLVTVSSGGGGSGGGGSGGGGSGGGGSQSVLTQPPSASGTPGQRVTISCSGGASNIETNYVSWYQQLPGTAPKLLIYDNNRRPSGVPDRFSGSKSGTSASLAISGLRSEDEADYYCAAWDDSLNGVIFGGGTKLTVL

SEQ ID NO: 48 - DNA, 750 bp, synthetic construct
  source 1..750: mol_type = other DNA
gaagtgcagctgctggaatctggcggaggactggttcaacctggcggctctctgagactgtcttgtgccgccagcggcttcacctttagcagctatggcatccactgggtccgacaggcccctggcaaaggacttgaatgggtcgccgtgattccctacgacggcagcaacaagtactacgccgacagcgtgaagggcagattcaccatcagccgggacaacagcaagaacaccctgtacctgcagatgaacagcctgagagccgaggacaccgccgtgtactactgtgccagagatccctggggctacgactacggactggatgtttggggccagggcacactggtcacagtttctagcggaggcggaggttctggcggcggaggaagtggtggcggaggctcaggtggcggtggatctcaatctgtgctgacccagcctcctagcgcctctggaacacctggacagagagtgaccatcagctgtagcggcggagccagcaacatcgagacaaactacgtgtcctggtatcagcagctccccggcacagctcccaaactgctgatctacgacaacaacagacggcccagcggcgtgcccgatagattttctggcagcaagagcggcacctctgccagcctggctatctctggactgagaagcgaggacgaggccgactattactgtgccgcctgggacgatagcctgaacggcgttatatttggaggcggcaccaagctgaccgtgctg

SEQ ID NO: 49 - protein, 5 aa, synthetic construct
SYGMH

SEQ ID NO: 50 - protein, 17 aa, synthetic construct
VIPYDGSNKYYADSVKG

SEQ ID NO: 51 - protein, 11 aa, synthetic construct
DPWGYDYGLDV

SEQ ID NO: 52 - protein, 13 aa, synthetic construct
SGGASNIGSNYVS

SEQ ID NO: 53 - protein, 7 aa, synthetic construct
DNNQRPS

SEQ ID NO: 54 - protein, 11 aa, synthetic construct
AAWDDSLSGVV

SEQ ID NO: 55 - protein, 120 aa, synthetic construct
QVQLVESGGGVVQPGGSLRLSCAASGFTFSSYGMHWVRQAPGKGLEWVAVIPYDGSNKYYADSVKGRFTISRDNSKNTLYLQMNSLRAEDTAVYYCARDPWGYDYGLDVWGQGTTVTVSS

SEQ ID NO: 56 - protein, 110 aa, synthetic construct
QSVLTQPPSASGTPGQRVTISCSGGASNIGSNYVSWYQQLPGTAPKLLIYDNNQRPSGVPDRFSGSKSGTSASLAISGLRSEDEADYYCAAWDDSLSGVVFGGGTKLTVL

SEQ ID NO: 57 - protein, 250 aa, synthetic construct
QVQLVESGGGVVQPGGSLRLSCAASGFTFSSYGMHWVRQAPGKGLEWVAVIPYDGSNKYYADSVKGRFTISRDNSKNTLYLQMNSLRAEDTAVYYCARDPWGYDYGLDVWGQGTTVTVSSGGGGSGGGGSGGGGSGGGGSQSVLTQPPSASGTPGQRVTISCSGGASNIGSNYVSWYQQLPGTAPKLLIYDNNQRPSGVPDRFSGSKSGTSASLAISGLRSEDEADYYCAAWDDSLSGVVFGGGTKLTVL

SEQ ID NO: 58 - DNA, 750 bp, synthetic construct
  source 1..750: mol_type = other DNA
caggtgcagctggttgaatctggtggcggagttgttcagcctggcggctctctgagactgtcttgtgccgccagcggcttcacctttagcagctatggcatgcactgggtccgacaggcccctggcaaaggacttgaatgggtcgccgtgattccctacgacggcagcaacaagtactacgccgacagcgtgaagggcagattcaccatcagccgggacaacagcaagaacaccctgtacctgcagatgaacagcctgagagccgaggacaccgccgtgtactactgtgccagagatccctggggctacgactacggactggatgtttggggccagggcaccaccgtgacagtttctagcggaggcggaggaagtggcggcggaggatctggcggtggtggtagtggcggtggcggttctcaatctgtgctgacacagcctcctagcgcctctggaacacctggacagagagtgaccatcagctgtagcggcggagccagcaacatcggcagcaattacgtgtcctggtatcagcagctgcccggcacagctcccaaactgctgatctacgacaacaaccagcggcctagcggcgtgcccgatagattttctggcagcaagagcggcacctctgccagcctggctatctctggactgagaagcgaggacgaggccgactattactgtgccgcctgggatgatagcctgtccggcgttgtgtttggcggaggcacaaagctgacagtgctg

SEQ ID NO: 59 - protein, 5 aa, synthetic construct
DHYMD

SEQ ID NO: 60 - protein, 17 aa, synthetic construct
VIWYDGSNKYYADSVKG

SEQ ID NO: 61 - protein, 12 aa, synthetic construct
RPRGYYYYGMDV

SEQ ID NO: 62 - protein, 13 aa, synthetic construct
SGGSSNIGSNPVN

SEQ ID NO: 63 - protein, 7 aa, synthetic construct
GNTQRPS

SEQ ID NO: 64 - protein, 11 aa, synthetic construct
AAWDDSLSGWV

SEQ ID NO: 65 - protein, 121 aa, synthetic construct
QVQLVESGGGLVQPGGSLRLSCAASGFTFSDHYMDWVRQAPGKGLEWVAVIWYDGSNKYYADSVKGRFTISRDNSKNTLYLQMNSLRAEDTAVYYCARRPRGYYYYGMDVWGQGTLVTVSS

SEQ ID NO: 66 - protein, 110 aa, synthetic construct
QSVLTQPPSASGTPGQRVTISCSGGSSNIGSNPVNWYQQLPGTAPKLLIYGNTQRPSGVPDRFSGSKSGTSASLAISGLRSEDEADYYCAAWDDSLSGWVFGGGTKLTVL

SEQ ID NO: 67 - protein, 251 aa, synthetic construct
QVQLVESGGGLVQPGGSLRLSCAASGFTFSDHYMDWVRQAPGKGLEWVAVIWYDGSNKYYADSVKGRFTISRDNSKNTLYLQMNSLRAEDTAVYYCARRPRGYYYYGMDVWGQGTLVTVSSGGGGSGGGGSGGGGSGGGGSQSVLTQPPSASGTPGQRVTISCSGGSSNIGSNPVNWYQQLPGTAPKLLIYGNTQRPSGVPDRFSGSKSGTSASLAISGLRSEDEADYYCAAWDDSLSGWVFGGGTKLTVL

SEQ ID NO: 68 - DNA, 753 bp, synthetic construct
  source 1..753: mol_type = other DNA
caggtgcagctggttgaatctggcggaggactggttcagcctggcggatctctgagactgtcttgtgccgccagcggcttcaccttcagcgaccactatatggactgggtccgacaggcccctggcaaaggacttgaatgggtcgccgtgatttggtacgacggcagcaacaagtactacgccgacagcgtgaagggcagattcaccatcagccgggacaacagcaagaacaccctgtacctgcagatgaacagcctgagagccgaggacaccgccgtgtactattgtgccagaaggcccagaggctactactactatggcatggacgtgtggggccagggcacactggttacagtttctagcggaggcggaggttctggcggcggaggaagtggtggcggaggctcaggtggcggtggatctcaatctgtgctgacccagcctcctagcgcctctggaacacctggacagagagtgaccatcagctgtagcggcggcagcagcaacatcggcagcaatcccgtgaactggtatcagcagctgcctggcacagcccctaaactgctgatctacggcaacacccagaggcctagcggcgtgccagatagattttccggcagcaagagcggcaccagcgcttctctggctatcagcggactgagaagcgaggacgaggccgattattactgcgccgcctgggatgatagcctgagcggatgggttttcggcggaggcacaaagctgacagtgctg

SEQ ID NO: 69 - protein, 5 aa, synthetic construct
DHYMD

SEQ ID NO: 70 - protein, 17 aa, synthetic construct
VIWYDGSNKYYADSVKG

SEQ ID NO: 71 - protein, 12 aa, synthetic construct
RPRGYYYYGTDV

SEQ ID NO: 72 - protein, 13 aa, synthetic construct
SGGSSNIGSNPVN

SEQ ID NO: 73 - protein, 7 aa, synthetic construct
GNTQRPS

SEQ ID NO: 74 - protein, 11 aa, synthetic construct
AAWDDSLSGWV

SEQ ID NO: 75 - protein, 121 aa, synthetic construct
QVQLVESGGGLVQPGGSLRLSCAASGFTFSDHYMDWVRQAPGKGLEWVAVIWYDGSNKYYADSVKGRFTISRDNSKNTLYLQMNSLRAEDTAVYYCARRPRGYYYYGTDVWGQGTLVTVSS

SEQ ID NO: 76 - protein, 110 aa, synthetic construct; identical to SEQ ID NO: 66

SEQ ID NO: 77 - protein, 251 aa, synthetic construct
QVQLVESGGGLVQPGGSLRLSCAASGFTFSDHYMDWVRQAPGKGLEWVAVIWYDGSNKYYADSVKGRFTISRDNSKNTLYLQMNSLRAEDTAVYYCARRPRGYYYYGTDVWGQGTLVTVSSGGGGSGGGGSGGGGSGGGGSQSVLTQPPSASGTPGQRVTISCSGGSSNIGSNPVNWYQQLPGTAPKLLIYGNTQRPSGVPDRFSGSKSGTSASLAISGLRSEDEADYYCAAWDDSLSGWVFGGGTKLTVL

SEQ ID NO: 78 - DNA, 753 bp, synthetic construct
  source 1..753: mol_type = other DNA
caggtgcagctggttgaatctggcggaggactggttcagcctggcggatctctgagactgtcttgtgccgccagcggcttcaccttcagcgaccactatatggactgggtccgacaggcccctggcaaaggacttgaatgggtcgccgtgatttggtacgacggcagcaacaagtactacgccgacagcgtgaagggcagattcaccatcagccgggacaacagcaagaacaccctgtacctgcagatgaacagcctgagagccgaggacaccgccgtgtactattgtgccagaaggcccagaggctactactactatggcaccgatgtgtggggccagggcacactggttacagtttctagcggaggcggaggttctggcggcggaggaagtggtggcggaggctcaggtggcggtggatctcaatctgtgctgacccagcctcctagcgcctctggaacacctggacagagagtgaccatcagctgtagcggcggcagcagcaacatcggcagcaatcccgtgaactggtatcagcagctgcctggcacagcccctaaactgctgatctacggcaacacccagaggcctagcggcgtgccagatagattttccggcagcaagagcggcaccagcgcttctctggctatcagcggactgagaagcgaggacgaggccgattattactgcgccgcctgggatgatagcctgagcggatgggttttcggcggaggcacaaagctgacagtgctg

SEQ ID NO: 79 - protein, 5 aa, synthetic construct
TYYLH

SEQ ID NO: 80 - protein, 17 aa, synthetic construct
WIYPGNVHAQYNEKFKG

SEQ ID NO: 81 - protein, 7 aa, synthetic construct
SWEGFPY

SEQ ID NO: 82 - protein, 11 aa, synthetic construct
KASQNVGINVA

SEQ ID NO: 83 - protein, 7 aa, synthetic construct
SASYRYS

SEQ ID NO: 84 - protein, 9 aa, synthetic construct
QQYDTYPFT

SEQ ID NO: 85 - protein, 240 aa, synthetic construct
QVQLVQSGAEVKKPGSSVKVSCKASGYTFTTYYLHWVRQAPGCGLEWMGWIYPGNVHAQYNEKFKGRVTITADKSTSTAYMELSSLRSEDTAVYYCARSWEGFPYWGQGTTVTVSSGGGSGGGSGCPPCGGGGDIQMTQSPSSLSASVGDRVTITCKASQNVGINVAWYQQKPGKAPKSLISSASYRYSGVPSRFSGSGSGTDFTLTISSLQPEDFATYFCQQYDTYPFTFGCGTKVEIK

SEQ ID NO: 86 - protein, 711 aa, synthetic construct
EVQLLESGGGLVQPGGSLRLSCAASGFTFSNYAMHWVRQAPGKGLEWVSAISGSGGSTYYADSVKGRFTISRDNSKNTLYLQMNSLRAEDTAVYYCARGRLPDVWGQGTLVTVSSASTKGPSVFPLAPSSKSTSGGTAALGCLVKDYFPEPVTVSWNSGALTSGVHTFPAVLQSSGLYSLSSVVTVPSSSLGTQTYICNVNHKPSNTKVDKKVEPKSCDKTHTCPPCPAPEAAGGPSVFLFPPKPKDTLMISRTPEVTCVVVDVSHEDPEVKFNWYVDGVEVHNAKTKPREEQYNSTYRVVSVLTVLHQDWLNGKEYKCKVSNKALPAPIEKTISKAKGQPREPQVYTLPPSRDELTKNQVSLTCLVKGFYPSDIAVEWESNGQPENNYKTTPPVLDSDGSFFLYSKLTVDKSRWQQGNVFSCSVMHEALHNHYTQKSLSLSPGGGGGSGGSGGSGGGGGQVQLVESGGGLVQPGGSLRLSCAASGFTFSDHYMDWVRQAPGKGLEWVAVIWYDGSNKYYADSVKGRFTISRDNSKNTLYLQMNSLRAEDTAVYYCARRPRGYYYYGTDVWGQGTLVTVSSGGGGSGGGGSGGGGSGGGGSQSVLTQPPSASGTPGQRVTISCSGGSSNIGSNPVNWYQQLPGTAPKLLIYGNTQRPSGVPDRFSGSKSGTSASLAISGLRSEDEADYYCAAWDDSLSGWVFGGGTKLTVL

SEQ ID NO: 87 - protein, 216 aa, synthetic construct
QSVLTQPPSASGTPGQRVTISCSGSSSNIGNNYVSWYQQLPGTAPKLLIYSNNQRPAGVPDRFSGSKSGTSASLAISGLRSEDEADYYCAAWDDSLNGGVFGGGTKLTVLGQPKAAPSVTLFPPSSEELQANKATLVCLISDFYPGAVTVAWKADSSPVKAGVETTTPSKQSNNKYAASSYLSLTPEQWKSHRSYSCQVTHEGSTVEKTVAPTECS

SEQ ID NO: 88 - protein, 710 aa, synthetic construct
EVQLLESGGGLVQPGGSLRLSCAASGFTFSNYAMHWVRQAPGKGLEWVSAISGSGGSTYYADSVKGRFTISRDNSKNTLYLQMNSLRAEDTAVYYCARGRLPDVWGQGTLVTVSSASTKGPSVFPLAPSSKSTSGGTAALGCLVKDYFPEPVTVSWNSGALTSGVHTFPAVLQSSGLYSLSSVVTVPSSSLGTQTYICNVNHKPSNTKVDKKVEPKSCDKTHTCPPCPAPPVAGPSVFLFPPKPKDTLMISRTPEVTCVVVGVSHEDPEVKFNWYVDGVEVHNAKTKPREEQYNSTYRVVSVLTVLHQDWLNGKEYKCKVSNKQLPSPIEKTISKAKGQPREPQVYTLPPSRDELTKNQVSLTCLVKGFYPSDIAVEWESNGQPENNYKTTPPVLDSDGSFFLYSKLTVDKSRWQQGNVFSCSVMHEALHNHYTQKSLSLSPGGGGGSGGSGGSGGGGGQVQLVESGGGLVQPGGSLRLSCAASGFTFSDHYMDWVRQAPGKGLEWVAVIWYDGSNKYYADSVKGRFTISRDNSKNTLYLQMNSLRAEDTAVYYCARRPRGYYYYGTDVWGQGTLVTVSSGGGGSGGGGSGGGGSGGGGSQSVLTQPPSASGTPGQRVTISCSGGSSNIGSNPVNWYQQLPGTAPKLLIYGNTQRPSGVPDRFSGSKSGTSASLAISGLRSEDEADYYCAAWDDSLSGWVFGGGTKLTVL

SEQ ID NO: 89 - protein, 216 aa, synthetic construct; identical to SEQ ID NO: 87

SEQ ID NO: 90 - protein, 706 aa, synthetic construct
EVQLLESGGGLVQPGGSLRLSCAASGFTFSNYAMHWVRQAPGKGLEWVSAISGSGGSTYYADSVKGRFTISRDNSKNTLYLQMNSLRAEDTAVYYCARGRLPDVWGQGTLVTVSSAKTTPPSVYPLAPGSAAQTNSMVTLGCLVKGYFPEPVTVTWNSGSLSSGVHTFPAVLQSDLYTLSSSVTVPSSTWPSETVTCNVAHPASSTKVDKKIVPRDCGCKPCICTVPEVSSVFIFPPKPKDVLTITLTPKVTCVVVDISKDDPEVQFSWFVDDVEVHTAQTQPREEQFASTFRSVSELPIMHQDWLNGKEFKCRVNSAAFPAPIEKTISKTKGRPKAPQVYTIPPPKEQMAKDKVSLTCMITDFFPEDITVEWQWNGQPAENYKNTQPIMDTDGSYFVYSKLNVQKSNWEAGNTFTCSVLHEGLHNHHTEKSLSHSPGKGGGGSGGSGGSGGGGGQVQLVESGGGLVQPGGSLRLSCAASGFTFSDHYMDWVRQAPGKGLEWVAVIWYDGSNKYYADSVKGRFTISRDNSKNTLYLQMNSLRAEDTAVYYCARRPRGYYYYGTDVWGQGTLVTVSSGGGGSGGGGSGGGGSGGGGSQSVLTQPPSASGTPGQRVTISCSGGSSNIGSNPVNWYQQLPGTAPKLLIYGNTQRPSGVPDRFSGSKSGTSASLAISGLRSEDEADYYCAAWDDSLSGWVFGGGTKLTVL

SEQ ID NO: 91 - protein, 216 aa, synthetic construct
QSVLTQPPSASGTPGQRVTISCSGSSSNIGNNYVSWYQQLPGTAPKLLIYSNNQRPAGVPDRFSGSKSGTSASLAISGLRSEDEADYYCAAWDDSLNGGVFGGGTKLTVLGQPKSSPSVTLFPPSSEELETNKATLVCTITDFYPGVVTVDWKVDGTPVTQGMETTQPSKQSNNKYMASSYLTLTARAWERHSSYSCQVTHEGHTVEKSLSRADCS

SEQ ID NO: 92 - protein, 706 aa, synthetic construct
EVQLLESGGGLVQPGGSLRLSCAASGFTFSNYAMHWVRQAPGKGLEWVSAISGSGGSTYYADSVKGRFTISRDNSKNTLYLQMNSLRAEDTAVYYCARGRLPDVWGQGTLVTVSSAKTTPPSVYPLAPGSAAQTNSMVTLGCLVKGYFPEPVTVTWNSGSLSSGVHTFPAVLQSDLYTLSSSVTVPSSTWPSETVTCNVAHPASSTKVDKKIVPRDCGCKPCICTVPEVSSVFIFPPKPKDVLTITLTPKVTCVVVDISKDDPEVQFSWFVDDVEVHTAQTQPREEQFASTFRSVSELPIMHQDWLNGKEFKCRVNSAAFPAPIEKTISKTKGRPKAPQVYTIPPPKEQMAKDKVSLTCMITDFFPEDITVEWQWNGQPAENYKNTQPIMDTDGSYFVYSKLNVQKSNWEAGNTFTCSVLHEGLHNHHTEKSLSHSPGKGGGGSGGSGGSGGGGGEVQLLESGGGLVQPGGSLRLSCAASGFTFSDHYMDWVRQAPGKGLEWVAVIWYDGSNKYYADSVKGRFTISRDNSKNTLYLQMNSLRAEDTAVYYCARRPRGYYYYGMDVWGQGTLVTVSSGGGGSGGGGSGGGGSGGGGSQSVLTQPPSASGTPGQRVTISCSGGSSNVGSNPVNWYQQLPGTAPKLLIYGNTNRPSGVPDRFSGSKSGTSASLAISGLRSEDEADYYCAAWDASLSGWVFGGGTKLTVL

SEQ ID NO: 93 - protein, 216 aa, synthetic construct; identical to SEQ ID NO: 91

SEQ ID NO: 94 - protein, 439 aa, synthetic construct
EVQLLESGGGLVQPGGSLRLSCAASGFTFSNYAMHWVRQAPGKGLEWVSAISGSGGSTYYADSVKGRFTISRDNSKNTLYLQMNSLRAEDTAVYYCARGRLPDVWGQGTLVTVSSAKTTPPSVYPLAPGSAAQTNSMVTLGCLVKGYFPEPVTVTWNSGSLSSGVHTFPAVLQSDLYTLSSSVTVPSSTWPSETVTCNVAHPASSTKVDKKIVPRDCGCKPCICTVPEVSSVFIFPPKPKDVLTITLTPKVTCVVVDISKDDPEVQFSWFVDDVEVHTAQTQPREEQFASTFRSVSELPIMHQDWLNGKEFKCRVNSAAFPAPIEKTISKTKGRPKAPQVYTIPPPKEQMAKDKVSLTCMITDFFPEDITVEWQWNGQPAENYKNTQPIMDTDGSYFVYSKLNVQKSNWEAGNTFTCSVLHEGLHNHHTEKSLSHSPGK

SEQ ID NO: 95 - protein, 467 aa, synthetic construct
QSVLTQPPSASGTPGQRVTISCSGSSSNIGNNYVSWYQQLPGTAPKLLIYSNNQRPAGVPDRFSGSKSGTSASLAISGLRSEDEADYYCAAWDDSLNGGVFGGGTKLTVLGQPKAAPSVTLFPPSSEELQANKATLVCLISDFYPGAVTVAWKADSSPVKAGVETTTPSKQSNNKYAASSYLSLTPEQWKSHRSYSCQVTHEGSTVEKTVAPTECSGEVQLLESGGGLVQPGGSLRLSCAASGFTFSDHYMDWVRQAPGKGLEWVAVIWYDGSNKYYADSVKGRFTISRDNSKNTLYLQMNSLRAEDTAVYYCARRPRGYYYYGMDVWGQGTLVTVSGGGGSGGGGSGGGGSGGGGSQSVLTQPPSASGTPGQRVTISCSGGSSNVGSNPVNWYQQLPGTAPKLLIYGNTNRPSGVPDRFSGSKSGTSASLAISGLRSEDEADYYCAAWDASLSGWVFGGGTKLTVL

SEQ ID NO: 96 - protein, 710 aa, synthetic construct
EVQLLESGGGLVQPGGSLRLSCAASGFTFSNYAMHWVRQAPGKGLEWVSAISGSGGSTYYADSVKGRFTISRDNSKNTLYLQMNSLRAEDTAVYYCARGRLPDVWGQGTLVTVSSASTKGPSVFPLAPSSKSTSGGTAALGCLVKDYFPEPVTVSWNSGALTSGVHTFPAVLQSSGLYSLSSVVTVPSSSLGTQTYICNVNHKPSNTKVDKKVEPKSCDKTHTCPPCPAPPVAGPSVFLFPPKPKDTLMISRTPEVTCVVVGVSHEDPEVKFNWYVDGVEVHNAKTKPREEQYNSTYRVVSVLTVLHQDWLNGKEYKCKVSNKQLPSPIEKTISKAKGQPREPQVYTLPPSRDELTKNQVSLTCLVKGFYPSDIAVEWESNGQPENNYKTTPPVLDSDGSFFLYSKLTVDKSRWQQGNVFSCSVMHEALHNHYTQKSLSLSPGGGGGSGGSGGSGGGGGEVQLLESGGGLVQPGGSLRLSCAASGFTFSDHYMDWVRQAPGKGLEWVAVIWYDGSNKYYADSVKGRFTISRDNSKNTLYLQMNSLRAEDTAVYYCARRPRGYYYYGMDVWGQGTLVTVSSGGGGSGGGGSGGGGSGGGGSQSVLTQPPSASGTPGQRVTISCSGGSSNVGSNPVNWYQQLPGTAPKLLIYGNTNRPSGVPDRFSGSKSGTSASLAISGLRSEDEADYYCAAWDASLSGWVFGGGTKLTVL

SEQ ID NO: 97 - protein, 216 aa, synthetic construct; identical to SEQ ID NO: 87

SEQ ID NO: 98 - protein, 711 aa, synthetic construct
EVQLLESGGGLVQPGGSLRLSCAASGFTFSNYAMHWVRQAPGKGLEWVSAISGSGGSTYYADSVKGRFTISRDNSKNTLYLQMNSLRAEDTAVYYCARGRLPDVWGQGTLVTVSSASTKGPSVFPLAPSSKSTSGGTAALGCLVKDYFPEPVTVSWNSGALTSGVHTFPAVLQSSGLYSLSSVVTVPSSSLGTQTYICNVNHKPSNTKVDKKVEPKSCDKTHTCPPCPAPELLGGPSVFLFPPKPKDTLMISRTPEVTCVVVDVSHEDPEVKFNWYVDGVEVHNAKTKPREEQYNSTYRVVSVLTVLHQDWLNGKEYKCKVSNKALPAPIEKTISKAKGQPREPQVYTLPPSRDELTKNQVSLTCLVKGFYPSDIAVEWESNGQPENNYKTTPPVLDSDGSFFLYSKLTVDKSRWQQGNVFSCSVMHEALHNHYTQKSLSLSPGGGGGSGGSGGSGGGGGEVQLLESGGGLVQPGGSLRLSCAASGFTFSDHYMDWVRQAPGKGLEWVAVIWYDGSNKYYADSVKGRFTISRDNSKNTLYLQMNSLRAEDTAVYYCARRPRGYYYYGMDVWGQGTLVTVSSGGGGSGGGGSGGGGSGGGGSQSVLTQPPSASGTPGQRVTISCSGGSSNVGSNPVNWYQQLPGTAPKLLIYGNTNRPSGVPDRFSGSKSGTSASLAISGLRSEDEADYYCAAWDASLSGWVFGGGTKLTVL

SEQ ID NO: 99 - protein, 216 aa, synthetic construct; identical to SEQ ID NO: 87

SEQ ID NO: 100 - protein, 708 aa, synthetic construct
EVQLLESGGGLVQPGGSLRLSCAASGFTFSNYAMHWVRQAPGKGLEWVSAISGSGGSTYYADSVKGRFTISRDNSKNTLYLQMNSLRAEDTAVYYCARGRLPDVWGQGTLVTVSSASTKGPSVFPLAPCSRSTSESTAALGCLVKDYFPEPVTVSWNSGALTSGVHTFPAVLQSSGLYSLSSVVTVPSSSLGTKTYTCNVDHKPSNTKVDKRVESKYGPPCPPCPAPEFLGGPSVFLFPPKPKDTLMISRTPEVTCVVVDVSQEDPEVQFNWYVDGVEVHNAKTKPREEQFNSTYRVVSVLTVLHQDWLNGKEYKCKVSNKGLPSSIEKTISKAKGQPREPQVYTLPPSQEEMTKNQVSLTCLVKGFYPSDIAVEWESNGQPENNYKTTPPVLDSDGSFFLYSRLTVDKSRWQEGNVFSCSVMHEALHNHYTQKSLSLSLGGGGGSGGSGGSGGGGGEVQLLESGGGLVQPGGSLRLSCAASGFTFSDHYMDWVRQAPGKGLEWVAVIWYDGSNKYYADSVKGRFTISRDNSKNTLYLQMNSLRAEDTAVYYCARRPRGYYYYGMDVWGQGTLVTVSSGGGGSGGGGSGGGGSGGGGSQSVLTQPPSASGTPGQRVTISCSGGSSNVGSNPVNWYQQLPGTAPKLLIYGNTNRPSGVPDRFSGSKSGTSASLAISGLRSEDEADYYCAAWDASLSGWVFGGGTKLTVL

SEQ ID NO: 101 - protein, 216 aa, synthetic construct; identical to SEQ ID NO: 87

SEQ ID NO: 102 - protein, 711 aa, synthetic construct
EVQLLESGGGLVQPGGSLRLSCAASGFTFSNYAMHWVRQAPGKGLEWVSAISGSGGSTYYADSVKGRFTISRDNSKNTLYLQMNSLRAEDTAVYYCARGRLPDVWGQGTLVTVSSASTKGPSVFPLAPSSKSTSGGTAALGCLVKDYFPEPVTVSWNSGALTSGVHTFPAVLQSSGLYSLSSVVTVPSSSLGTQTYICNVNHKPSNTKVDKKVEPKSCDKTHTCPPCPAPEAAGASSVFLFPPKPKDTLMISRTPEVTCVVVDVSAEDPEVKFNWYVDGVEVHNAKTKPREEQYNSTYRVVSVLTVLHQDWLNGKEYKCKVSNKALPSSIEKTISKAKGQPREPQVYTLPPSREEMTKNQVSLTCLVKGFYPSDIAVEWESNGQPENNYKTTPPVLDSDGSFFLYSKLTVDKSRWQQGNVFSCSVMHEALHNHYTQKSLSLSPGKGGGGSGGGGSGGGGSQVQLVESGGGLVQPGGSLRLSCAASGFTFSDHYMDWVRQAPGKGLEWVAVIWYDGSNKYYADSVKGRFTISRDNSKNTLYLQMNSLRAEDTAVYYCARRPRGYYYYGMDVWGQGTLVTVSSGGGGSGGGGSGGGGSGGGGSQSVLTQPPSASGTPGQRVTISCSGGSSNIGSNPVNWYQQLPGTAPKLLIYGNTQRPSGVPDRFSGSKSGTSASLAISGLRSEDEADYYCAAWDDSLSGWVFGGGTKLTVL

SEQ ID NO: 103 - protein, 216 aa, synthetic construct; identical to SEQ ID NO: 87

SEQ ID NO: 104 - protein, 715 aa, synthetic construct
QVQLQQSGPELEKPGASVKISCKASGYSFTGYTMNWVKQSHGKSLEWIGLITPYNGASSYNQKFRGKATLTVDKSSSTAYMDLLSLTSEDSAVYFCARGGYDGRGFDYWGSGTPVTVSSASTKGPSVFPLAPSSKSTSGGTAALGCLVKDYFPEPVTVSWNSGALTSGVHTFPAVLQSSGLYSLSSVVTVPSSSLGTQTYICNVNHKPSNTKVDKKVEPKSCDKTHTCPPCPAPEAAGASSVFLFPPKPKDTLMISRTPEVTCVVVDVSAEDPEVKFNWYVDGVEVHNAKTKPREEQYNSTYRVVSVLTVLHQDWLNGKEYKCKVSNKALPSSIEKTISKAKGQPREPQVYTLPPSREEMTKNQVSLTCLVKGFYPSDIAVEWESNGQPENNYKTTPPVLDSDGSFFLYSKLTVDKSRWQQGNVFSCSVMHEALHNHYTQKSLSLSPGKGGGGSGGGGSGGGGSQVQLVESGGGLVQPGGSLRLSCAASGFTFSDHYMDWVRQAPGKGLEWVAVIWYDGSNKYYADSVKGRFTISRDNSKNTLYLQMNSLRAEDTAVYYCARRPRGYYYYGMDVWGQGTLVTVSSGGGGSGGGGSGGGGSGGGGSQSVLTQPPSASGTPGQRVTISCSGGSSNIGSNPVNWYQQLPGTAPKLLIYGNTQRPSGVPDRFSGSKSGTSASLAISGLRSEDEADYYCAAWDDSLSGWVFGGGTKLTVL

SEQ ID NO: 105 - protein, 213 aa, synthetic construct
DIELTQSPAIMSASPGEKVTMTCSASSSVSYMHWYQQKSGTSPKRWIYDTSKLASGVPGRFSGSGSGNSYSLTISSVEAEDDATYYCQQWSKHPLTFGSGTKVEIKRTVAAPSVFIFPPSDEQLKSGTASVVCLLNNFYPREAKVQWKVDNALQSGNSQESVTEQDSKDSTYSLSSTLTLSKADYEKHKVYACEVTHQGLSSPVTKSFNRGEC

SEQ ID NO: 106 - protein, 700 aa, synthetic construct
EVQLLESGGGLVQPGGSLRLSCAASGFTFSNYAMHWVRQAPGKGLEWVSAISGSGGSTYYADSVKGRFTISRDNSKNTLYLQMNSLRAEDTAVYYCARGRLPDVWGQGTLVTVSSASTKGPSVFPLAPSSKSTSGGTAALGCLVKDYFPEPVTVSWNSGALTSGVHTFPAVLQSSGLYSLSSVVTVPSSSLGTQTYICNVNHKPSNTKVDKKVEPKSCDKTHTCPPCPAPEAAGASSVFLFPPKPKDTLMISRTPEVTCVVVDVSAEDPEVKFNWYVDGVEVHNAKTKPREEQYNSTYRVVSVLTVLHQDWLNGKEYKCKVSNKALPSSIEKTISKAKGQPREPQVYTLPPSREEMTKNQVSLTCLVKGFYPSDIAVEWESNGQPENNYKTTPPVLDSDGSFFLYSKLTVDKSRWQQGNVFSCSVMHEALHNHYTQKSLSLSPGKGGGGSGGGGSGGGGSQVQLVQSGAEVKKPGSSVKVSCKASGYTFTTYYLHWVRQAPGCGLEWMGWIYPGNVHAQYNEKFKGRVTITADKSTSTAYMELSSLRSEDTAVYYCARSWEGFPYWGQGTTVTVSSGGGSGGGSGCPPCGGGGDIQMTQSPSSLSASVGDRVTITCKASQNVGINVAWYQQKPGKAPKSLISSASYRYSGVPSRFSGSGSGTDFTLTISSLQPEDFATYFCQQYDTYPFTFGCGTKVEIK

SEQ ID NO: 107 - protein, 216 aa, synthetic construct; identical to SEQ ID NO: 87

SEQ ID NO: 108 - protein, 704 aa, synthetic construct
QVQLQQSGPELEKPGASVKISCKASGYSFTGYTMNWVKQSHGKSLEWIGLITPYNGASSYNQKFRGKATLTVDKSSSTAYMDLLSLTSEDSAVYFCARGGYDGRGFDYWGSGTPVTVSSASTKGPSVFPLAPSSKSTSGGTAALGCLVKDYFPEPVTVSWNSGALTSGVHTFPAVLQSSGLYSLSSVVTVPSSSLGTQTYICNVNHKPSNTKVDKKVEPKSCDKTHTCPPCPAPEAAGASSVFLFPPKPKDTLMISRTPEVTCVVVDVSAEDPEVKFNWYVDGVEVHNAKTKPREEQYNSTYRVVSVLTVLHQDWLNGKEYKCKVSNKALPSSIEKTISKAKGQPREPQVYTLPPSREEMTKNQVSLTCLVKGFYPSDIAVEWESNGQPENNYKTTPPVLDSDGSFFLYSKLTVDKSRWQQGNVFSCSVMHEALHNHYTQKSLSLSPGKGGGGSGGGGSGGGGSQVQLVQSGAEVKKPGSSVKVSCKASGYTFTTYYLHWVRQAPGCGLEWMGWIYPGNVHAQYNEKFKGRVTITADKSTSTAYMELSSLRSEDTAVYYCARSWEGFPYWGQGTTVTVSSGGGSGGGSGCPPCGGGGDIQMTQSPSSLSASVGDRVTITCKASQNVGINVAWYQQKPGKAPKSLISSASYRYSGVPSRFSGSGSGTDFTLTISSLQPEDFATYFCQQYDTYPFTFGCGTKVEIK

SEQ ID NO: 109 - protein, 213 aa, synthetic construct; identical to SEQ ID NO: 105

SEQ ID NO: 110 - protein, 213 aa, synthetic construct
DIQMTQSPDSLSASVGDRVTITCRASQDVGSWLAWYQQKPGKAPKLLIFAASYLESGIPSRFSGSGSGTDFTLTISSLQPEDFATYYCQQANGFPLTFGGGTKVEIKRTVAAPSVFIFPPSDEQLKSGTASVVCLLNNFYPREAKVQWKVDNALQSGNSQESVTEQDSKDSTYSLSSTLTLSKADYEKHKVYACEVTHQGLSSPVTKSFNRGE

SEQ ID NO: 111 - protein, 712 aa, synthetic construct
EVQLLESGGGLVQPGGSLRLSCAASGFTFSGYMMSWVRQAPGKGLEWVSGIYPSPGYTYYADSVKGRFTISRDNSKNTLYLQMNSLRAEDTAVYYCAREKASDLSGSYSEALDYWGQGTLVTVSSASTKGPSVFPLAPCSRSTSESTAALGCLVKDYFPEPVTVSWNSGALTSGVHTFPAVLQSSGLYSLSSVVTVPSSNFGTQTYTCNVDHKPSNTKVDKTVERKCCVECPPCPAPPVAGPSVFLFPPKPKDTLMISRTPEVTCVVVDVSHEDPEVQFNWYVDGVEVHNAKTKPREEQFNSTFRVVSVLTVVHQDWLNGKEYKCKVSNKGLPAPIEKTISKTKGQPREPQVYTLPPSREEMTKNQVSLTCLVKGFYPSDIAVEWESNGQPENNYKTTPPMLDSDGSFFLYSKLTVDKSRWQQGNVFSCSVMHEALHNHYTQKSLSLSPGGGGGSGGSGGSGGGGGEVQLLESGGGLVQPGGSLRLSCAASGFTFSSYSMNWVRQAPGKGLEWVSYITGSSGTTYYADSVKGRFTISRDNSKNTLYLQMNSLRAEDTAVYYCARGGWSLDYWGQGTLVTVSSGGGGSGGGGSGGGGSGGGGSQSVLTQPPSASGTPGQRVTISCSGSTSNIGFNYVYWYQQLPGTAPKLLIYGNNNRPSGVPDRFSGSKSGTSASLTISGLRSEDEADYYCAAWDDSLSGRVFGGGTKLTVL

SEQ ID NO: 112 - protein, 444 aa, synthetic construct
EVQLLESGGGLVQPGGSLRLSCAASGFTFSNYAMHWVRQAPGKGLEWVSAISGSGGSTYYADSVKGRFTISRDNSKNTLYLQMNSLRAEDTAVYYCARGRLPDVWGQGTLVTVSSASTKGPSVFPLAPSSKSTSGGTAALGCLVKDYFPEPVTVSWNSGALTSGVHTFPAVLQSSGLYSLSSVVTVPSSSLGTQTYICNVNHKPSNTKVDKKVEPKSCDKTHTCPPCPAPELLGGPSVFLFPPKPKDTLMISRTPEVTCVVVDVSHEDPEVKFNWYVDGVEVHNAKTKPREEQYNSTYRVVSVLTVLHQDWLNGKEYKCKVSNKALPAPIEKTISKAKGQPREPQVYTLPPSRDELTKNQVSLTCLVKGFYPSDIAVEWESNGQPENNYKTTPPVLDSDGSFFLYSKLTVDKSRWQQGNVFSCSVMHEALHNHYTQKSLSLSPG

SEQ ID NO: 113 - protein, 216 aa, synthetic construct; identical to SEQ ID NO: 87

SEQ ID NO: 114 - protein, 439 aa, synthetic construct; identical to SEQ ID NO: 94

SEQ ID NO: 115 - protein, 216 aa, synthetic construct; identical to SEQ ID NO: 91

SEQ ID NO: 116 - protein, 450 aa, synthetic construct
QVQLKQSGPGLVQPSQSLSLTCTVSGFSLTSYGVHWVRQPPGKGLEWLGVIWSGGSTDYNAAFISRLSIRKDNSKSQVFFKMNSLQADDTAIYYCARTFTTSTSAWFAYWGQGTLVTVSAASTKGPSVFPLAPSSKSTSGGTAALGCLVKDYFPEPVTVSWNSGALTSGVHTFPAVLQSSGLYSLSSVVTVPSSSLGTQTYICNVNHKPSNTKVDKKVEPKSCDKTHTCPPCPAPELLGGPSVFLFPPKPKDTLMISRTPEVTCVVVDVSHEDPEVKFNWYVDGVEVHNAKTKPREEQYNSTYRVVSVLTVLHQDWLNGKEYKCKVSNKALPAPIEKTISKAKGQPREPQVYTLPPSRDELTKNQVSLTCLVKGFYPSDIAVEWESNGQPENNYKTTPPVLDSDGSFFLYSKLTVDKSRWQQGNVFSCSVMHEALHNHYTQKSLSLSPGK

SEQ ID NO: 117 - protein, 215 aa, synthetic construct
SIVMTQTPKFLLVSAGDRVTITCKASQSVSNDVAWYQQKPGQSPKLLIYYASNRYTGVPDRFTGSGYGTDFTFTISTVQAEDLAVYFCQQDYSSPPWTFGGGTKLEIRRTVAAPSVFIFPPSDEQLKSGTASVVCLLNNFYPREAKVQWKVDNALQSGNSQESVTEQDSKDSTYSLSSTLTLSKADYEKHKVYACEVTHQGLSSPVTKSFNRGEC

SEQ ID NO: 118 - protein, 621 aa, synthetic construct
QETELSVSAELVPTSSWNISSELNKDSYLTLDEPMNNITTSLGQTAELHCKVSGNPPPTIRWFKNDAPVVQEPRRLSFRSTIYGSRLRIRNLDTTDTGYFQCVATNGKEVVSSTGVLFVKFGPPPTASPGYSDEYEEDGFCQPYRGIACARFIGNRTVYMESLHMQGEIENQITAAFTMIGTSSHLSDKCSQFAIPSLCHYAFPYCDETSSVPKPRDLCRDECEILENVLCQTEYIFARSNPMILMRLKLPNCEDLPQPESPEAANCIRIGIPMADPINKNHKCYNSTGVDYRGTVSVTKSGRQCQPWNSQYPHTHTFTALRFPELNGGHSYCRNPGNQKEAPWCFTLDENFKSDLCDIPACDSKDSKEKNKMEGGGSIEGRMDPKSCDKTHTCPPCPAPELLGGPSVFLFPPKPKDTLMISRTPEVTCVVVDVSHEDPEVKFNWYVDGVEVHNAKTKPREEQYNSTYRVVSVLTVLHQDWLNGKEYKCKVSNKALPAPIEKTISKAKGQPREPQVYTLPPSREEMTKNQVSLTCLVKGFYPSDIAVEWESNGQPENNYKTTPPVLDSDGSFFLYSKLTVDKSRWQQGNVFSCSVMHEALHNHYTQKSLSLSPGKHHHHHH

SEQ ID NO: 119 - protein, 454 aa, synthetic construct
EVQLLESGGGLVQPGGSLRLSCAASGFTFSGYMMQWVRQAPGKGLEWVSGIYPSGGYTNYADSVKGRFTISRDNSKNTLYLQMNSLRAEDTATYYCAREKASDLSGSYSEALDYWGQGTLVTVSSASTKGPSVFPLAPSSKSTSGGTAALGCLVKDYFPEPVTVSWNSGALTSGVHTFPAVLQSSGLYSLSSVVTVPSSSLGTQTYICNVNHKPSNTKVDKKVEPKSCDKTHTCPPCPAPELLGGPSVFLFPPKPKDTLMISRTPEVTCVVVDVSHEDPEVKFNWYVDGVEVHNAKTKPREEQYNSTYRVVSVLTVLHQDWLNGKEYKCKVSNKALPAPIEKTISKAKGQPREPQVYTLPPSRDELTKNQVSLTCLVKGFYPSDIAVEWESNGQPENNYKTTPPVLDSDGSFFLYSKLTVDKSRWQQGNVFSCSVMHEALHNHYTQKSLSLSPG

SEQ ID NO: 120 - protein, 216 aa, synthetic construct
AQDIQMTQSPDSLSASVGDRVTITCRASQDVGSWLAWYQQKPGKAPKLLIFAASSLESGIPSRFSGSGSGTDFTLTISSLQPEDFATYYCQQANGFPLTFGGGTKVEIKRTVAAPSVFIFPPSDEQLKSGTASVVCLLNNFYPREAKVQWKVDNALQSGNSQESVTEQDSKDSTYSLSSTLTLSKADYEKHKVYACEVTHQGLSSPVTKSFNRGEC

SEQ ID NO: 121 - protein, 120 aa, synthetic construct
EVQLVQSGAEVKKPGASVKVSCKASGYKFSSYWIEWVKQAPGQGLEWIGEILPGSDTTNYNEKFKDRATFTSDTSINTAYMELSRLRSDDTAVYYCARDRGNYRAWFGYWGQGTLVTVSS

SEQ ID NO: 122 - protein, 5 aa, synthetic construct
SYWIE

SEQ ID NO: 123 - protein, 17 aa, synthetic construct
EILPGSDTTNYNEKFKD

SEQ ID NO: 124 - protein, 11 aa, synthetic construct
DRGNYRAWFGY

SEQ ID NO: 125 - protein, 107 aa, synthetic construct
DIQMTQSPSSLSASVGDRVTITCRASQSISSYLNWYQQKPGGAPKFLIYYASSLQSGVPSRFSGSGSGTDYTLTISSLQPEDFATYYCQQGFSLPWTFGGGTKVEIK

SEQ ID NO: 126 - protein, 11 aa, synthetic construct
RASQSISSYLN

SEQ ID NO: 127 - protein, 7 aa, synthetic construct
YASSLQS

SEQ ID NO: 128 - protein, 9 aa, synthetic construct
QQGFSLPWT

SEQ ID NO: 129 - DNA, 360 bp, synthetic construct
  source 1..360: mol_type = other DNA
gaggtgcagctggtgcagtctggcgccgaagtgaaaaagcctggcgcctctgtgaaggtgtcctgcaaggcttccggctacaagttctccagctactggatcgagtgggtcaagcaggctcctggacagggactcgagtggatcggagagatcctgcctggctctgacaccaccaactacaacgagaagttcaaggaccgggccaccttcacctccgacacctctatcaacaccgcctacatggaactgtcccggctgagatctgacgacaccgccgtgtactactgcgccagagacagaggcaactacagagcttggtttggctactggggccagggcacactggttacagttagctca

SEQ ID NO: 130 - DNA, 321 bp, synthetic construct
  source 1..321: mol_type = other DNA
gatatccagatgacccagtctccttccagcctgtctgcctctgtgggcgacagagtgaccatcacctgtcgggcctctcagtccatctcctcctacctgaactggtatcagcagaagcctggcggcgctcccaagttcctgatctactacgctagctccctgcagtccggcgtgccctctagattttctggctctggatccggcaccgactataccctgacaatctccagcctgcagcctgaggacttcgccacctactattgccagcagggcttctccctgccttggacatttggcggcggaacaaaggtggaaatcaaa

SEQ ID NO: 131 - protein, 449 aa, synthetic construct
EVQLVQSGAEVKKPGASVKVSCKASGYKFSSYWIEWVKQAPGQGLEWIGEILPGSDTTNYNEKFKDRATFTSDTSINTAYMELSRLRSDDTAVYYCARDRGNYRAWFGYWGQGTLVTVSSASTKGPSVFPLAPSSKSTSGGTAALGCLVKDYFPEPVTVSWNSGALTSGVHTFPAVLQSSGLYSLSSVVTVPSSSLGTQTYICNVNHKPSNTKVDKKVEPKSCDKTHTCPPCPAPELLGGPSVFLFPPKPKDTLMISRTPEVTCVVVDVSHEDPEVKFNWYVDGVEVHNAKTKPREEQYNSTYRVVSVLTVLHQDWLNGKEYKCKVSNKALPAPIEKTISKAKGQPREPQVYTLPPSRDELTKNQVSLTCLVKGFYPSDIAVEWESNGQPENNYKTTPPVLDSDGSFFLYSKLTVDKSRWQQGNVFSCSVMHEALHNHYTQKSLSLSPG

SEQ ID NO: 132 - protein, 214 aa, synthetic construct; identical to SEQ ID NO: 2

SEQ ID NO: 133 - protein, 454 aa, synthetic construct
EVQLLESGGGLVQPGGSLRLSCAASGFTFSGYMMSWVRQAPGKGLEWVSGIYPSPGYTYYADSVKGRFTISRDNSKNTLYLQMNSLRAEDTAVYYCAREKASDLFGSYSEALDYWGQGTLVTVSSASTKGPSVFPLAPSSKSTSGGTAALGCLVKDYFPEPVTVSWNSGALTSGVHTFPAVLQSSGLYSLSSVVTVPSSSLGTQTYICNVNHKPSNTKVDKKVEPKSCDKTHTCPPCPAPELLGGPSVFLFPPKPKDTLMISRTPEVTCVVVDVSHEDPEVKFNWYVDGVEVHNAKTKPREEQYNSTYRVVSVLTVLHQDWLNGKEYKCKVSNKALPAPIEKTISKAKGQPREPQVYTLPPSRDELTKNQVSLTCLVKGFYPSDIAVEWESNGQPENNYKTTPPVLDSDGSFFLYSKLTVDKSRWQQGNVFSCSVMHEALHNHYTQKSLSLSPG

SEQ ID NO: 134 - protein, 214 aa, synthetic construct
DIQMTQSPDSLSASVGDRVTITCRASQDVGSWLAWYQQKPGKAPKLLIFAASSLESGIPSRFSGSGSGTDFTLTISSLQPEDFATYYCQQANGFPLTFGGGTKVEIKRTVAAPSVFIFPPSDEQLKSGTASVVCLLNNFYPREAKVQWKVDNALQSGNSQESVTEQDSKDSTYSLSSTLTLSKADYEKHKVYACEVTHQGLSSPVTKSFNRGEC

SEQ ID NO: 135 - protein, 454 aa, synthetic construct
EVQLLESGGGLVQPGGSLRLSCAASGFTFSGYMMSWVRQAPGKGLEWVSGIYPSPGYTYYADSVKGRFTISRDNSKNTLYLQMNSLRAEDTAVYYCAREKASDLSGSYSEALDYWGQGTLVTVSSASTKGPSVFPLAPSSKSTSGGTAALGCLVKDYFPEPVTVSWNSGALTSGVHTFPAVLQSSGLYSLSSVVTVPSSSLGTQTYICNVNHKPSNTKVDKKVEPKSCDKTHTCPPCPAPELLGGPSVFLFPPKPKDTLMISRTPEVTCVVVDVSHEDPEVKFNWYVDGVEVHNAKTKPREEQYNSTYRVVSVLTVLHQDWLNGKEYKCKVSNKALPAPIEKTISKAKGQPREPQVYTLPPSRDELTKNQVSLTCLVKGFYPSDIAVEWESNGQPENNYKTTPPVLDSDGSFFLYSKLTVDKSRWQQGNVFSCSVMHEALHNHYTQKSLSLSPG

SEQ ID NO: 136 - protein, 214 aa, synthetic construct
DIQMTQSPDSLSASVGDRVTITCRASQDVGSWLAWYQQKPGKAPKLLIFAASYLESGIPSRFSGSGSGTDFTLTISSLQPEDFATYYCQQANGFPLTFGGGTKVEIKRTVAAPSVFIFPPSDEQLKSGTASVVCLLNNFYPREAKVQWKVDNALQSGNSQESVTEQDSKDSTYSLSSTLTLSKADYEKHKVYACEVTHQGLSSPVTKSFNRGEC

SEQ ID NO: 137 - protein, 454 aa, synthetic construct
EVQLLESGGGLVQPGGSLRLSCAASGFTFSGYMMSWVRQAPGKGLEWVSGIYPSGGYALYADSVKGRFTISRDNSKNTLYLQMNSLRAEDTAVYYCAREKAADLFGSYSEALDYWGQGTLVTVSSASTKGPSVFPLAPSSKSTSGGTAALGCLVKDYFPEPVTVSWNSGALTSGVHTFPAVLQSSGLYSLSSVVTVPSSSLGTQTYICNVNHKPSNTKVDKKVEPKSCDKTHTCPPCPAPELLGGPSVFLFPPKPKDTLMISRTPEVTCVVVDVSHEDPEVKFNWYVDGVEVHNAKTKPREEQYNSTYRVVSVLTVLHQDWLNGKEYKCKVSNKALPAPIEKTISKAKGQPREPQVYTLPPSRDELTKNQVSLTCLVKGFYPSDIAVEWESNGQPENNYKTTPPVLDSDGSFFLYSKLTVDKSRWQQGNVFSCSVMHEALHNHYTQKSLSLSPG

SEQ ID NO: 138 - protein, 214 aa, synthetic construct; identical to SEQ ID NO: 136

SEQ ID NO: 139 - protein, 120 aa, synthetic construct
EVQLVQSGAEVKKPGASVKVSCKASGYKFSSYWIEWVKQAPGQGLEWIGEILPGSDWTNYNEKFKDRATFTSDTSINTAYMELSRLRSDDTAVYYCARDRGNYRAWFQYWGQGTLVTVSS

SEQ ID NO: 140 - protein, 5 aa, synthetic construct
SYWIE

SEQ ID NO: 141 - protein, 17 aa, synthetic construct
EILPGSDWTNYNEKFKD

SEQ ID NO: 142 - protein, 11 aa, synthetic construct
DRGNYRAWFQY

SEQ ID NO: 143 - protein, 107 aa, synthetic construct
DIQMTQSPSSLSASVGDRVTITCRASQSISSYLNWYQQKPGGAPKFLIYYASSLQSGVPSRFSGSGSGTDYTLTISSLQPEDFATYYCQQGLELPWTFGGGTKVEIK

SEQ ID NO: 144 - protein, 11 aa, synthetic construct
RASQSISSYLN

SEQ ID NO: 145 - protein, 7 aa, synthetic construct
YASSLQS

SEQ ID NO: 146 - protein, 9 aa, synthetic construct
QQGLELPWT

SEQ ID NO: 147 - DNA, 360 bp, synthetic construct
  source 1..360: mol_type = other DNA
gaggtgcagctggtgcagtctggcgccgaagtgaaaaagcctggcgcctctgtgaaggtgtcctgcaaggcttccggctacaagttctccagctactggatcgagtgggtcaagcaggctcctggacagggactcgagtggatcggagagatcctgcctggctctgactggaccaactacaacgagaagttcaaggaccgggccaccttcacctccgacacctctatcaacaccgcctacatggaactgtcccggctgagatctgacgacaccgccgtgtactactgcgccagagacagaggcaactacagagcctggtttcagtactggggccagggcacactggtcacagtttcttca

SEQ ID NO: 148 - DNA, 321 bp, synthetic construct
  source 1..321: mol_type = other DNA
gatatccagatgacccagtctccttccagcctgtctgcctctgtgggcgacagagtgaccatcacctgtcgggcctctcagtccatctcctcctacctgaactggtatcagcagaagcctggcggcgctcccaagttcctgatctactacgctagctccctgcagtccggcgtgccctctagattttctggctctggatccggcaccgactataccctgacaatctccagcctgcagcctgaggacttcgccacctactactgtcagcagggactcgagctgccctggacatttggcggaggcaccaaggtggaaatcaaa

SEQ ID NO: 149 - protein, 449 aa, synthetic construct
EVQLVQSGAEVKKPGASVKVSCKASGYKFSSYWIEWVKQAPGQGLEWIGEILPGSDWTNYNEKFKDRATFTSDTSINTAYMELSRLRSDDTAVYYCARDRGNYRAWFQYWGQGTLVTVSSASTKGPSVFPLAPSSKSTSGGTAALGCLVKDYFPEPVTVSWNSGALTSGVHTFPAVLQSSGLYSLSSVVTVPSSSLGTQTYICNVNHKPSNTKVDKKVEPKSCDKTHTCPPCPAPELLGGPSVFLFPPKPKDTLMISRTPEVTCVVVDVSHEDPEVKFNWYVDGVEVHNAKTKPREEQYNSTYRVVSVLTVLHQDWLNGKEYKCKVSNKALPAPIEKTISKAKGQPREPQVYTLPPSRDELTKNQVSLTCLVKGFYPSDIAVEWESNGQPENNYKTTPPVLDSDGSFFLYSKLTVDKSRWQQGNVFSCSVMHEALHNHYTQKSLSLSPG

SEQ ID NO: 150 - protein, 214 aa, synthetic construct; identical to SEQ ID NO: 22

SEQ ID NO: 151 - protein, 449 aa, synthetic construct; identical to SEQ ID NO: 131

SEQ ID NO: 152 - protein, 214 aa, synthetic construct
DIQMTQSPSSLSASVGDRVTITCRASQDISNYLNWYQQKPGGAVKFLIYYTSRLHSGVPSRFSGSGSGTDYTLTISSLQPEDFATYFCQQGEALPWTFGGGTKVEIKRTVAAPSVFIFPPSDEQLKSGTASVVCLLNNFYPREAKVQWKVDNALQSGNSQESVTEQDSKDSTYSLSSTLTLSKADYEKHKVYACEVTHQGLSSPVTKSFNRGEC